European Patent Application EP 4 368 195 A1, published May 15, 2024. Title: Novel combinations of antibiotics and non-antibiotic drugs effective in vivo against Gram-positive bacteria, in particular methicillin-resistant S. aureus (MRSA). Applicant: European Molecular Biology Laboratory. Application EP. The sequence listing filed with the application follows.

SEQUENCE LISTING (3 sequences)

SEQ ID NO: 1 - RNA, 20 nt, S. aureus Newman
  source 1..20: mol_type = other RNA
tgtctaacagcaatgctttg

SEQ ID NO: 2 - RNA, 20 nt, S. aureus Newman
  source 1..20: mol_type = other RNA
aaaccataatttgcataaca

SEQ ID NO: 3 - RNA, 20 nt, S. aureus Newman
  source 1..20: mol_type = other RNA
atagaggatagaatggcgcc